European Patent Specification EP 4 103 693 B1, published December 3, 2025. Title: Fleischerzeugung in vitro. Applicant: Leibnitz-Institut für Nutztierbiologie. The sequence listing filed with the application follows.

SEQUENCE LISTING (16 sequences)

SEQ ID NO: 1 - DNA, 20 bp, Sus scrofa
cgtggcgcgactttctacca

SEQ ID NO: 2 - DNA, 20 bp, Sus scrofa
ccagggccatggcatcgtaa

SEQ ID NO: 3 - DNA, 24 bp, Sus scrofa
tcgctctcttgctaacagtcttgc

SEQ ID NO: 4 - DNA, 21 bp, Sus scrofa
ctgaatgggcaggttggtggt

SEQ ID NO: 5 - DNA, 20 bp, Sus scrofa
tcagcaacgaggtggtcgtc

SEQ ID NO: 6 - DNA, 20 bp, Sus scrofa
ccacgtcaggccccagattc

SEQ ID NO: 7 - DNA, 22 bp, Sus scrofa
tcgacaccgagactgtctctcc

SEQ ID NO: 8 - DNA, 20 bp, Sus scrofa
acagagctgggtctgcgaga

SEQ ID NO: 9 - DNA, 20 bp, Sus scrofa
cccgccctatgacttctgcg

SEQ ID NO: 10 - DNA, 20 bp, Sus scrofa
ctgggactcctcggggttcg

SEQ ID NO: 11 - DNA, 20 bp, Sus scrofa
cagtggtcaagtccgaggcg

SEQ ID NO: 12 - DNA, 20 bp, Sus scrofa
tgtaccgttgatggccgtgc

SEQ ID NO: 13 - DNA, 20 bp, Sus scrofa
tgccaaatagacgacgaaga

SEQ ID NO: 14 - DNA, 21 bp, Sus scrofa
acgacacattacggagtctga

SEQ ID NO: 15 - DNA, 21 bp, Sus scrofa
tgaaacctcactgcctgctgc

SEQ ID NO: 16 - DNA, 22 bp, Sus scrofa
agggtcttcgcccagcctttct